European Patent Specification EP 3 983 559 B1, published April 29, 2026. Title: In-situ concatenation of oligo-nucleotide probes for target detection. Applicant: QBiotix Limited. The sequence listing filed with the application follows.

SEQUENCE LISTING (120 sequences)

SEQ ID NO: 1 - DNA, 42 bp, Artificial Sequence
  Probe Sequence 3h
cgtgaagtcttttggtgcataaaatgtctgcttttatactaa

SEQ ID NO: 2 - DNA, 34 bp, Artificial Sequence
  DNA Target Sequence 3
tagtataaaagcagacattttatgcaccaaaaga

SEQ ID NO: 3 - DNA, 41 bp, Artificial Sequence
  Probe Sequence 4e
ccgcatgtcctgtgggtcctgaaacattgcagttccttcac

SEQ ID NO: 4 - DNA, 28 bp, Artificial Sequence
  DNA Target Sequence 4
gaactgcaatgtttcaggacccacagga

SEQ ID NO: 5 - DNA, 42 bp, Artificial Sequence
  Probe Sequence 5f
ggcgcctgcataactgtggtaactttctgggtcgccatgcgg

SEQ ID NO: 6 - DNA, 28 bp, Artificial Sequence
  DNA Target Sequence 5
gcgacccagaaagttaccacagttatgc

SEQ ID NO: 7 - DNA, 47 bp, Artificial Sequence
  Probe Sequence 6k
accgtcaaatattatatcatgtatagttgtttgcagctctgggcgcc

SEQ ID NO: 8 - DNA, 35 bp, Artificial Sequence
  DNA Target Sequence 6
acagagctgcaaacaactatacatgatataatatt

SEQ ID NO: 9 - DNA, 45 bp, Artificial Sequence
  Probe Sequence 7h
tcccctacagtaactgttgcttgcagtacacacattcttgacggt

SEQ ID NO: 10 - DNA, 31 bp, Artificial Sequence
  DNA Target Sequence 7
agaatgtgtgtactgcaagcaacagttactg

SEQ ID NO: 11 - DNA, 43 bp, Artificial Sequence
  Probe Sequence 8d
ggcttgccgaaaagcaaagtcatatacctcacgtcgtagggga

SEQ ID NO: 12 - DNA, 29 bp, Artificial Sequence
  DNA Target Sequence 8
cgacgtgaggtatatgactttgcttttcg

SEQ ID NO: 13 - DNA, 42 bp, Artificial Sequence
  Probe Sequence 9e
atggattcccatctctatatactatgcataaatccgcaagcc

SEQ ID NO: 14 - DNA, 35 bp, Artificial Sequence
  DNA Target Sequence 9
ggatttatgcatagtatatagagatgggaatccat

SEQ ID NO: 15 - DNA, 43 bp, Artificial Sequence
  Probe 3g
tcttttggtgcataaaatgtctgcttttatactaaaggtcatg

SEQ ID NO: 16 - DNA, 43 bp, Artificial Sequence
  Probe 4d
tgaccttcctgtgggtcctgaaacattgcagttcaatcaaact

SEQ ID NO: 17 - DNA, 46 bp, Artificial Sequence
  Probe 5e
agtttgatttgcataactgtggtaactttctgggtcgcactctagt

SEQ ID NO: 18 - DNA, 46 bp, Artificial Sequence
  Probe 6j
tctagagtaatattatatcatgtatagttgtttgcagctctgcatg

SEQ ID NO: 19 - DNA, 39 bp, Artificial Sequence
  Probe 7f
catgcagtaactgttgcttgcagtacacacattcccgcg

SEQ ID NO: 20 - DNA, 40 bp, Artificial Sequence
  Probe 8c
cgcggcgaaaagcaaagtcatatacctcacgtcgagacgg

SEQ ID NO: 21 - DNA, 47 bp, Artificial Sequence
  Probe 9d
ccgtctatggattcccatctctatatactatgcataaatccaagggg

SEQ ID NO: 22 - DNA, 19 bp, Artificial Sequence
  Probe Sequence 10
catttatcacatacagcat

SEQ ID NO: 23 - DNA, 19 bp, Artificial Sequence
  DNA Target Sequence 10
atgctgtatgtgataaatg

SEQ ID NO: 24 - DNA, 41 bp, Artificial Sequence
  Probe Sequence c1b
acgcgcataaagtgtatgtcgtatacctaagggtagagata

SEQ ID NO: 25 - DNA, 34 bp, Artificial Sequence
  DNA Target Sequence c1b
tatctctacccttaggtatacgacatacactatt

SEQ ID NO: 26 - DNA, 52 bp, Artificial Sequence
  Probe Sequence c2b
ggtactgcatattgatacgtatttagggcttttcgtttcagtatatgcgcgt

SEQ ID NO: 27 - DNA, 37 bp, Artificial Sequence
  DNA Target Sequence c2b
catatactgaaacgaaaagccctaaatacgtatcata

SEQ ID NO: 28 - DNA, 47 bp, Artificial Sequence
  Probe Sequence c3b
gtgggtacagtgcagcgtcattgacaacgaacgtcatgtgcagtacc

SEQ ID NO: 29 - DNA, 31 bp, Artificial Sequence
  DNA Target Sequence c3b
catgacgttcgttgtcaatgacgctgcactc

SEQ ID NO: 30 - DNA, 53 bp, Artificial Sequence
  Probe Sequence c4b
ccagggagtgtgtaagattataatatagtacatatcaacaaacgtgtacccac

SEQ ID NO: 31 - DNA, 37 bp, Artificial Sequence
  DNA Target Sequence c4b
acgtttgttgatatgtactatattataatcttacaca

SEQ ID NO: 32 - DNA, 45 bp, Artificial Sequence
  Probe Sequence c5b
ccacggtaccgagacacgtattgacaccattgaaagactccctgg

SEQ ID NO: 33 - DNA, 28 bp, Artificial Sequence
  DNA Target Sequence c5b
tctttcaatggtgtcaatacgtgtctcg

SEQ ID NO: 34 - DNA, 47 bp, Artificial Sequence
  Probe Sequence c6b
ggtagggcccagcgaggacacccaggactttgtaagctgtaccgtgg

SEQ ID NO: 35 - DNA, 31 bp, Artificial Sequence
  DNA Target Sequence c6b
acgttacaaagtcctgggtgtcctcgctggg

SEQ ID NO: 36 - DNA, 39 bp, Artificial Sequence
  Probe Sequence c7b
caagagaaaaccacgtattttacagacgaaaaccctacc

SEQ ID NO: 37 - DNA, 32 bp, Artificial Sequence
  DNA Target Sequence c7b
ttttcgtctgtaaaatacgtggttttctcttg

SEQ ID NO: 38 - DNA, 17 bp, Artificial Sequence
  Half Target 3a
tagtataaaagcagaca

SEQ ID NO: 39 - DNA, 17 bp, Artificial Sequence
  Half Probe 3a'
tgtctgcttttatacta

SEQ ID NO: 40 - DNA, 17 bp, Artificial Sequence
  Half Target 3b
ttttatgcaccaaaaga

SEQ ID NO: 41 - DNA, 17 bp, Artificial Sequence
  Half Probe 3b'
tcttttggtgcataaaa

SEQ ID NO: 42 - DNA, 16 bp, Artificial Sequence
  Half Target 4a
gaactgcaatgtttca

SEQ ID NO: 43 - DNA, 16 bp, Artificial Sequence
  Half Probe 4a'
tgaaacattgcagttc

SEQ ID NO: 44 - DNA, 12 bp, Artificial Sequence
  Half Target 4b
ggacccacagga

SEQ ID NO: 45 - DNA, 12 bp, Artificial Sequence
  Half Probe 4b'
tcctgtgggtcc

SEQ ID NO: 46 - DNA, 12 bp, Artificial Sequence
  Half Target 5a
gcgacccagaaa

SEQ ID NO: 47 - DNA, 12 bp, Artificial Sequence
  Half Probe 5a'
tttctgggtcgc

SEQ ID NO: 48 - DNA, 16 bp, Artificial Sequence
  Half Target 5b
gttaccacagttatgc

SEQ ID NO: 49 - DNA, 16 bp, Artificial Sequence
  Half Probe 5b'
gcataactgtggtaac

SEQ ID NO: 50 - DNA, 14 bp, Artificial Sequence
  Half Target 6a
acagagctgcaaac

SEQ ID NO: 51 - DNA, 14 bp, Artificial Sequence
  Half Probe 6a'
gtttgcagctctgt

SEQ ID NO: 52 - DNA, 21 bp, Artificial Sequence
  Half Target 6b
aactatacatgatataatatt

SEQ ID NO: 53 - DNA, 21 bp, Artificial Sequence
  Half Probe 6b'
aatattatatcatgtatagtt

SEQ ID NO: 54 - DNA, 15 bp, Artificial Sequence
  Half Target 7a
agaatgtgtgtactg

SEQ ID NO: 55 - DNA, 14 bp, Artificial Sequence
  Half Probe 7a'
cagtacacacattc

SEQ ID NO: 56 - DNA, 16 bp, Artificial Sequence
  Half Target 7b
caagcaacagttactg

SEQ ID NO: 57 - DNA, 16 bp, Artificial Sequence
  Half Probe 7b'
cagtaactgttgcttg

SEQ ID NO: 58 - DNA, 14 bp, Artificial Sequence
  Half Target 8a
cgacgtgaggtata

SEQ ID NO: 59 - DNA, 14 bp, Artificial Sequence
  Half Probe 8a'
tatacctcacgtcg

SEQ ID NO: 60 - DNA, 15 bp, Artificial Sequence
  Half Target 8b
tgactttgcttttcg

SEQ ID NO: 61 - DNA, 15 bp, Artificial Sequence
  Half Probe 8b'
cgaaaagcaaagtca

SEQ ID NO: 62 - DNA, 18 bp, Artificial Sequence
  Half Target 9a
ggatttatgcatagtata

SEQ ID NO: 63 - DNA, 18 bp, Artificial Sequence
  Half Probe 9a'
tatactatgcataaatcc

SEQ ID NO: 64 - DNA, 17 bp, Artificial Sequence
  Half Target 9b
tagagatgggaatccat

SEQ ID NO: 65 - DNA, 17 bp, Artificial Sequence
  Half Probe 9b'
atggattcccatctcta

SEQ ID NO: 66 - DNA, 18 bp, Artificial Sequence
  Half Target 10a
atgctgtatgtgataaat

SEQ ID NO: 67 - DNA, 33 bp, Artificial Sequence
  Resulting cDNA Target (3b+4a)
ttttatgcaccaaaagagaactgcaatgtttca

SEQ ID NO: 68 - DNA, 33 bp, Artificial Sequence
  Resulting cDNA Probe 7'
tgaaacattgcagttctcttttggtgcataaaa

SEQ ID NO: 69 - DNA, 24 bp, Artificial Sequence
  Resulting cDNA Target (4b+5a)
ggacccacaggagcgacccagaaa

SEQ ID NO: 70 - DNA, 24 bp, Artificial Sequence
  Resulting cDNA Probe 6'
tttctgggtcgctcctgtgggtcc

SEQ ID NO: 71 - DNA, 30 bp, Artificial Sequence
  Resulting cDNA Target (5b+6a)
gttaccacagttatgcacagagctgcaaac

SEQ ID NO: 72 - DNA, 30 bp, Artificial Sequence
  Resulting cDNA Probe 5'
gtttgcagctctgtgcataactgtggtaac

SEQ ID NO: 73 - DNA, 36 bp, Artificial Sequence
  Resulting cDNA Target (6b+7a)
aactatacatgatataatattagaatgtgtgtactg

SEQ ID NO: 74 - DNA, 36 bp, Artificial Sequence
  Resulting cDNA Probe 4'
cagtacacacattctaatattatatcatgtatagtt

SEQ ID NO: 75 - DNA, 30 bp, Artificial Sequence
  Resulting cDNA Target (7b+8a)
caagcaacagttactgcgacgtgaggtata

SEQ ID NO: 76 - DNA, 30 bp, Artificial Sequence
  Resulting cDNA Probe 3'
tatacctcacgtcgcagtaactgttgcttg

SEQ ID NO: 77 - DNA, 33 bp, Artificial Sequence
  Resulting cDNA Target (8b+9a)
tgactttgcttttcgggatttatgcatagtata

SEQ ID NO: 78 - DNA, 33 bp, Artificial Sequence
  Resulting cDNA Probe 2'
tatactatgcataaatcccgaaaagcaaagtca

SEQ ID NO: 79 - DNA, 35 bp, Artificial Sequence
  Resulting cDNA Target (9b+10a)
tagagatgggaatccatatgctgtatgtgataaat

SEQ ID NO: 80 - DNA, 35 bp, Artificial Sequence
  Resulting cDNA Probe 1'
atttatcacatacagcatatggattcccatctcta

SEQ ID NO: 81 - DNA, 39 bp, Artificial Sequence
  Resulting cDNA Probes 7' with helping stems
accctgtgaaacattgcagttctcttttggtgcataaaa

SEQ ID NO: 82 - DNA, 38 bp, Artificial Sequence
  resulting cDNA Probes 6' with helping stems
tttgagggtttctgggtcgctcctgtgggtcccagggt

SEQ ID NO: 83 - DNA, 44 bp, Artificial Sequence
  Resulting cDNA Probes 5' with helping stems
ggatgtgtttgcagctctgtgcataactgtggtaacccctcaaa

SEQ ID NO: 84 - DNA, 47 bp, Artificial Sequence
  Resulting cDNA Probes 4' with helping stems
cgtcacagtacacacattctaatattatatcatgtatagttacccat

SEQ ID NO: 85 - DNA, 39 bp, Artificial Sequence
  Resulting cDNA Probes 3' with helping stems
cgcgtatacctcacgtcgcagtaactgttgcttgtgacg

SEQ ID NO: 86 - DNA, 47 bp, Artificial Sequence
  Resulting cDNA Probes 2' with helping stems
acgcgtatactatgcataaatcccgaaaagcaaagtcacgcgggttc

SEQ ID NO: 87 - DNA, 40 bp, Artificial Sequence
  Resulting cDNA Probes 1' with helping stems
atttatcacatacagcatatggattcccatctctacgcgt

SEQ ID NO: 88 - DNA, 21 bp, Artificial Sequence
  Staaur Probe Sequence
gcaagcttctcgtccgttcgc

SEQ ID NO: 89 - DNA, 21 bp, Artificial Sequence
  Staaur Target Sequence
gcgaacggacgagaagcttgc

SEQ ID NO: 90 - RNA, 22 nt, Artificial Sequence
  ß-lactamase gene TEM-1 #1 target
ugcugcaacuuuauccgccucc

SEQ ID NO: 91 - DNA, 40 bp, Artificial Sequence
  ß-lactamase gene TEM-1 #1 probe with stem
atgctgcatggaggcggataaagttgcagcaatgcagcat

SEQ ID NO: 92 - RNA, 25 nt, Artificial Sequence
  ß-lactamase gene TEM-1 #2 target
auccagucuauuaauuguugccggg

SEQ ID NO: 93 - DNA, 43 bp, Artificial Sequence
  ß-lactamase gene TEM-1 #2 probe with stem
atgctgcatcccggcaacaattaatagactggatatgcagcat

SEQ ID NO: 94 - RNA, 24 nt, Artificial Sequence
  ß-lactamase gene TEM-1 #3 target
aagcuagaguaaguaguucgccag

SEQ ID NO: 95 - DNA, 42 bp, Artificial Sequence
  ß-lactamase gene TEM-1 #3 probe with stem
atgctgcatctggcgaactacttactctagcttatgcagcat

SEQ ID NO: 96 - RNA, 26 nt, Artificial Sequence
  ß-lactamase gene TEM-1 #4 target
uuaauaguuugcgcaacguuguugcc

SEQ ID NO: 97 - DNA, 44 bp, Artificial Sequence
  ß-lactamase gene TEM-1 #4 probe with stem
atgctgcatggcaacaacgttgcgcaaactattaaatgcagcat

SEQ ID NO: 98 - RNA, 21 nt, Artificial Sequence
  ß-lactamase gene TEM-1 #5 target
auugcugcaggcaucguggug

SEQ ID NO: 99 - DNA, 39 bp, Artificial Sequence
  ß-lactamase gene TEM-1 #5 probe with stem
atgctgcatcaccacgatgcctgcagcaatatgcagcat

SEQ ID NO: 100 - RNA, 22 nt, Artificial Sequence
  ß-lactamase gene TEM-1 #6 target
ucacgcucgucguuugguaugg

SEQ ID NO: 101 - DNA, 40 bp, Artificial Sequence
  ß-lactamase gene TEM-1 #6 probe with stem
atgctgcatccataccaaacgacgagcgtgaatgcagcat

SEQ ID NO: 102 - RNA, 22 nt, Artificial Sequence
  ß-lactamase gene TEM-1 #7 target
cuucauucagcuccgguuccca

SEQ ID NO: 103 - DNA, 41 bp, Artificial Sequence
  ß-lactamase gene TEM-1 #7 probe with stem
atgctgcattgggaaccggagctgaatgaagaatgcagcat

SEQ ID NO: 104 - RNA, 24 nt, Artificial Sequence
  ß-lactamase gene TEM-1 #8 target
acgaucaaggcgaguuacaugauc

SEQ ID NO: 105 - DNA, 42 bp, Artificial Sequence
  ß-lactamase gene TEM-1 #8 probe with stem
atgctgcatgatcatgtaactcgccttgatcgtatgcagcat

SEQ ID NO: 106 - RNA, 23 nt, Artificial Sequence
  ß-lactamase gene TEM-1 #9 target
ccccauguugugcaaaaaagcgg

SEQ ID NO: 107 - DNA, 41 bp, Artificial Sequence
  ß-lactamase gene TEM-1 #9 probe with stem
atgctgcatccgcttttttgcacaacatggggatgcagcat

SEQ ID NO: 108 - RNA, 20 nt, Artificial Sequence
  ß-lactamase gene TEM-1 #10 target
uuagcuccuucgguccuccg

SEQ ID NO: 109 - DNA, 38 bp, Artificial Sequence
  ß-lactamase gene TEM-1 #10 probe with stem
atgctgcatcggaggaccgaaggagctaaatgcagcat

SEQ ID NO: 110 - DNA, 34 bp, Artificial Sequence
  Probe c1
taaagtgtatgtcgtatacctaagggtagagata

SEQ ID NO: 111 - DNA, 32 bp, Artificial Sequence
  Probe c2
acgtatttagggcttttcgtttcagtatatgg

SEQ ID NO: 112 - DNA, 28 bp, Artificial Sequence
  Probe c3
gtcattgacaacgaacgtcatgtgtgta

SEQ ID NO: 113 - DNA, 41 bp, Artificial Sequence
  Probe c4
tgtgtgtaagattataatatagtacatatcaacaaacgtcg

SEQ ID NO: 114 - DNA, 29 bp, Artificial Sequence
  Probe c5
agacacgtattgacaccattgaaagaccc

SEQ ID NO: 115 - DNA, 31 bp, Artificial Sequence
  Probe c6
agcgaggacacccaggactttgtaacaagag

SEQ ID NO: 116 - DNA, 33 bp, Artificial Sequence
  Probe c7
aaaaccacgtattttacagacgaaaatatgatt

SEQ ID NO: 117 - DNA, 37 bp, Artificial Sequence
  E. coli probe 5'-1 with stem: Atto-465
actcagtatctcgggagaaggcacgctgatactgagt

SEQ ID NO: 118 - DNA, 41 bp, Artificial Sequence
  E. coli probe with stem: Atto-514
actcagtacgcaagtcgcttcacctacatatcgtactgagt

SEQ ID NO: 119 - DNA, 41 bp, Artificial Sequence
  E. coli probe 3'+1 with stem: Atto-465
actcagtactggagctgaaatcagtcgaaggagtactgagt

SEQ ID NO: 120 - DNA, 64 bp, Escherichia coli
agcgtgccttctcccgagatatgtaggtgaagcgacttgctccttcgactgatttcagctccac